European Patent Application EP 4 375 289 A1, published May 29, 2024. Title: Peptide with antimicrrobial activity. Applicant: Freie Universität Berlin. The sequence listing filed with the application follows.

SEQUENCE LISTING (8 sequences)

SEQ ID NO: 1 - protein, 14 aa, synthetic construct
  SITE 2: note = 2-aminobutyric acid
  SITE 4: note = 2-aminobutyric acid
  SITE 8: note = 2-aminobenzoic acid
  SITE 11: note = 2-aminobutyric acid
  SITE 13: note = 2-aminobutyric acid
RXRXRLFXARXRXR

SEQ ID NO: 2 - protein, 14 aa, synthetic construct
  SITE 2: note = (2S)-4-monofluoroethylglycine
  SITE 4: note = (2S)-4-monofluoroethylglycine
  SITE 8: note = (2)-amino benzoic acid
  SITE 11: note = (2S)-4-monofluoroethylglycine
  SITE 13: note = (2S)-4-monofluoroethylglycine
RXRXRLFXARXRXR

SEQ ID NO: 3 - protein, 14 aa, synthetic construct
  SITE 2: note = (2S)-4,4-difluoroethylglycine
  SITE 4: note = (2S)-4,4-difluoroethylglycine
  SITE 8: note = 2-aminobenzoic acid
  SITE 11: note = (2S)-4,4-difluoroethylglycine
  SITE 13: note = (2S)-4,4-difluoroethylglycine
RXRXRLFXARXRXR

SEQ ID NO: 4 - protein, 14 aa, synthetic construct
  SITE 2: note = (2S)-4,4,4-trifluoroethylglycine
  SITE 4: note = (2S)-4,4,4-trifluoroethylglycine
  SITE 8: note = 2-aminobenzoic acid
  SITE 11: note = (2S)-4,4,4-trifluoroethylglycine
  SITE 13: note = (2S)-4,4,4-trifluoroethylglycine
RXRXRLFXARXRXR

SEQ ID NO: 5 - protein, 14 aa, synthetic construct
  SITE 8: note = 2-aminobenzoic acid
RVRWRLFXARWRVR

SEQ ID NO: 6 - protein, 14 aa, synthetic construct
  SITE 2: note = 2-aminobutyric acid
  SITE 8: note = 2-aminobenzoic acid
  SITE 13: note = 2-aminobutyric acid
RXRWRLFXARWRXR

SEQ ID NO: 7 - protein, 14 aa, synthetic construct
  SITE 2: note = (2S)-4,4,4-trifluoroethylglycine
  SITE 8: note = 2-aminobenzoic acid
  SITE 13: note = (2S)-4,4,4-trifluoroethylglycine
RXRWRLFXARWRXR

SEQ ID NO: 8 - protein, 14 aa, synthetic construct
  SITE 2: note = pentafluoropropylglycine
  SITE 8: note = 2-aminobenzoic acid
  SITE 13: note = pentafluoropropylglycine
RXRWRLFXARWRXR